European Patent Specification EP 3 804 736 B1, published November 19, 2025. Title: PHARMACEUTICAL COMPOSITION FOR PREVENTING OR TREATING INFLAMMATORY DISEASES COMPRISING MESENCHYMAL STEM CELLS. Applicant: MEDIPOST CO., LTD. The sequence listing filed with the application follows.

SEQUENCE LISTING (4 sequences)

SEQ ID NO: 1 - DNA, 21 bp, Artificial Sequence
  HLA-A2  siRNA (sense)
guucguguaggcauaaugutt

SEQ ID NO: 2 - DNA, 21 bp, Artificial Sequence
  HLA-A2  siRNA (anti-sense)
acauuaugccuacacgaactt

SEQ ID NO: 3 - DNA, 21 bp, Artificial Sequence
  control siRNA (sense)
ccuacgccaccaauuucgutt

SEQ ID NO: 4 - DNA, 21 bp, Artificial Sequence
  control siRNA (anti-sense)
acgaaauugguggcguaggtt